European Patent Application EP 4 653 453 A1, published November 26, 2025. Title: 痘病毒重组嵌合抗原、其亚单位疫苗及其应用. Applicant: 北京大学. The sequence listing filed with the application follows.

SEQUENCE LISTING (13 sequences)

SEQ ID NO: 1 - protein, 92 aa, synthetic construct
STTQYDHKESCNGLYYQGSCYILHSDYKSFEDAKANCAAESSTLPNKSDVLTTWLIDYVEDTWGSDGNPITKTTSDYQDSDVSQEVRKYFCT

SEQ ID NO: 2 - protein, 118 aa, synthetic construct
SANKAAITDSAVAVAAASSTHRKVVSSTTQYDHKESCNGLYYQGSCYILHSDYKSFEDAKANCAAESSTLPNKSDVLTTWLIDYVEDTWGSDGNPITKTTSDYQDSDVSQEVRKYFCT

SEQ ID NO: 3 - protein, 179 aa, synthetic construct
AAASIQTTVNTLSERISSKLEQEANASAQTKCDIEIGNFYIRQNHGCNITVKNMCSADADAQLDAVLSAATETYSGLTPEQKAYVPAMFTAALNIQTSVNTVVRDFENYVKQTCNSSAVVDNKLKIQNVIIDECYGAPGSPTNLEFINTGSSKGNCAIKALMQLTTKATTQIAPRQVAG

SEQ ID NO: 4 - protein, 568 aa, synthetic construct
STTQYDHKESCNGLYYQGSCYILHSDYKSFEDAKANCAAESSTLPNKSDVLTTWLIDYVEDTWGSDGNPITKTTSDYQDSDVSQEVRKYFCTAAASIQTTVNTLSERISSKLEQEANASAQTKCDIEIGNFYIRQNHGCNITVKNMCSADADAQLDAVLSAATETYSGLTPEQKAYVPAMFTAALNIQTSVNTVVRDFENYVKQTCNSSAVVDNKLKIQNVIIDECYGAPGSPTNLEFINTGSSKGNCAIKALMQLTTKATTQIAPRQVAGSANKAAITDSAVAVAAASSTHRKVVSSTTQYDHKESCNGLYYQGSCYILHSDYKSFEDAKANCAAESSTLPNKSDVLTTWLIDYVEDTWGSDGNPITKTTSDYQDSDVSQEVRKYFCTAAASIQTTVNTLSERISSKLEQEANASAQTKCDIEIGNFYIRQNHGCNITVKNMCSADADAQLDAVLSAATETYSGLTPEQKAYVPAMFTAALNIQTSVNTVVRDFENYVKQTCNSSAVVDNKLKIQNVIIDECYGAPGSPTNLEFINTGSSKGNCAIKALMQLTTKATTQIAPRQVAG

SEQ ID NO: 5 - protein, 20 aa, synthetic construct
METDTLLLWVLLLWVPGSTG

SEQ ID NO: 6 - protein, 594 aa, synthetic construct
METDTLLLWVLLLWVPGSTGSTTQYDHKESCNGLYYQGSCYILHSDYKSFEDAKANCAAESSTLPNKSDVLTTWLIDYVEDTWGSDGNPITKTTSDYQDSDVSQEVRKYFCTAAASIQTTVNTLSERISSKLEQEANASAQTKCDIEIGNFYIRQNHGCNITVKNMCSADADAQLDAVLSAATETYSGLTPEQKAYVPAMFTAALNIQTSVNTVVRDFENYVKQTCNSSAVVDNKLKIQNVIIDECYGAPGSPTNLEFINTGSSKGNCAIKALMQLTTKATTQIAPRQVAGSANKAAITDSAVAVAAASSTHRKVVSSTTQYDHKESCNGLYYQGSCYILHSDYKSFEDAKANCAAESSTLPNKSDVLTTWLIDYVEDTWGSDGNPITKTTSDYQDSDVSQEVRKYFCTAAASIQTTVNTLSERISSKLEQEANASAQTKCDIEIGNFYIRQNHGCNITVKNMCSADADAQLDAVLSAATETYSGLTPEQKAYVPAMFTAALNIQTSVNTVVRDFENYVKQTCNSSAVVDNKLKIQNVIIDECYGAPGSPTNLEFINTGSSKGNCAIKALMQLTTKATTQIAPRQVAGHHHHHH

SEQ ID NO: 7 - protein, 236 aa, synthetic construct
METDTLLLWVLLLWVPGSTGSTTQYDHKESCNGLYYQGSCYILHSDYKSFEDAKANCAAESSTLPNKSDVLTTWLIDYVEDTWGSDGNPITKTTSDYQDSDVSQEVRKYFCTSANKAAITDSAVAVAAASSTHRKVVSSTTQYDHKESCNGLYYQGSCYILHSDYKSFEDAKANCAAESSTLPNKSDVLTTWLIDYVEDTWGSDGNPITKTTSDYQDSDVSQEVRKYFCTHHHHHH

SEQ ID NO: 8 - protein, 181 aa, synthetic construct
MGAAASIQTTVNTLSERISSKLEQEANASAQTKCDIEIGNFYIRQNHGCNITVKNMCSADADAQLDAVLSAATETYSGLTPEQKAYVPAMFTAALNIQTSVNTVVRDFENYVKQTCNSSAVVDNKLKIQNVIIDECYGAPGSPTNLEFINTGSSKGNCAIKALMQLTTKATTQIAPRQVAG

SEQ ID NO: 9 - protein, 93 aa, synthetic construct
MSTTQYDHKESCNGLYYQGSCYILHSDYKSFEDAKANCAAESSTLPNKSDVLTTWLIDYVEDTWGSDGNPITKTTSDYQDSDVSQEVRKYFCT

SEQ ID NO: 10 - DNA, 1782 bp, synthetic construct
  source 1..1782: mol_type = other DNA
atggaaacagacaccctgctgctgtgggtcctgctgctctgggtgcctggcagcaccggcagcaccacccagtacgaccacaaagagagctgcaacggcctgtactaccaaggctcttgttacatcctgcacagcgactataagagcttcgaggatgctaaggccaattgcgccgccgagagcagcacactgcctaacaagtccgacgtgctgaccacctggctgatcgactacgtggaagatacatggggaagcgacggcaaccccatcacaaaaaccacaagcgattatcaggacagcgacgtgtctcaggaggttagaaagtacttttgcaccgccgccgcctctatccagaccacagtgaacaccctgagcgagcggatcagctccaagctggagcaggaggcaaacgcaagcgcccagacaaagtgcgacatcgagatcggcaatttctacatcagacagaaccacggctgcaatatcaccgtgaagaatatgtgctccgccgacgcagatgcacagctggatgccgtgctgtccgccgcaaccgagacatactctggcctgacccctgagcagaaggcctatgtgccagccatgttcacagccgccctgaacatccagaccagcgtgaatacagtggtgcgggactttgagaactacgtgaagcagacctgcaattctagcgccgtggtggacaacaagctgaagatccagaatgtgatcatcgatgagtgttatggagcaccaggatcccctaccaacctggagttcatcaatacaggctcctctaagggcaactgcgccatcaaggccctgatgcagctgaccacaaaggccaccacacagatcgcacctaggcaggtggcaggatccgccaataaggcagccatcaccgactctgccgtggcagtggcagcagccagctccacacaccgcaaggtggtgtctagcaccacacagtacgatcacaaggaatcctgtaatggcctgtactatcagggctcctgttacatcctgcactctgactataagagctttgaggatgccaaggccaactgtgccgccgagtcctctaccctgccaaataagagcgacgtgctgaccacatggctgatcgactatgtggaggatacctggggctctgatggcaaccccatcacaaagaccacatctgattaccaggacagcgacgtgagccaggaggtgcggaagtatttctgcaccgctgctgcttccatccagaccacagtgaatacactgagcgagagaatcagctccaaactggagcaggaggccaacgcctctgcccagaccaagtgtgacatcgagatcggcaacttctacatcaggcagaatcatggatgtaatatcaccgtgaagaacatgtgctccgccgatgccgacgcccagctggacgccgtgctgagcgccgccactgagacatactccggcctgacccccgaacagaaagcctatgtgcctgctatgtttaccgccgccctgaacattcagaccagcgtcaacacagtggtgcgcgatttcgaaaattatgtcaaacagacttgtaattctagcgccgtcgtcgataacaagctgaagattcagaatgtgattattgacgaatgctacggagcaccaggatccccaaccaacctggagtttatcaacaccggctcctctaagggcaattgtgccatcaaggccctgatgcaactgactaccaaagctaccacacagatcgcaccaaggcaggtggcaggacaccaccaccaccaccac

SEQ ID NO: 11 - DNA, 708 bp, synthetic construct
  source 1..708: mol_type = other DNA
atggaaacagacaccctgctgctgtgggtcctgctgctctgggtgcctggcagcaccggcagcaccacccagtacgaccacaaagagagctgcaacggcctgtactaccaaggctcttgttacatcctgcacagcgactataagagcttcgaggatgctaaggccaattgcgccgccgagagcagcacactgcctaacaagtccgacgtgctgaccacctggctgatcgactacgtggaagatacatggggaagcgacggcaaccccatcacaaaaaccacaagcgattatcaggacagcgacgtgtctcaggaggttagaaagtacttttgcaccagcgccaacaaagccgctatcaccgacagcgccgtggccgtggccgccgcatctagcacccacagaaaggtggtgtcctccacaacacagtacgaccacaaggaaagctgtaatggactgtactaccagggcagctgctacatcctgcacagcgactacaagtctttcgaggacgccaaggccaactgcgccgctgagtctagcaccctgccaaacaagagcgatgtgctgacaacctggctgattgactacgtggaagatacctggggctccgatggcaaccctatcaccaagaccacatctgactaccaggatagcgacgtgtcccaggaggtgcggaagtacttctgcacccaccaccaccaccaccat

SEQ ID NO: 12 - DNA, 543 bp, synthetic construct
  source 1..543: mol_type = other DNA
atgggagcagctgcgtcaatacaaacaactgtaaacaccctgagcgaacgtattagctccaaacttgagcaagaggcaaacgcgagcgcgcaaacgaaatgcgatattgagatcggcaacttctatatccgccaaaatcacggttgtaatattaccgtcaagaacatgtgcagcgcggacgcggacgcgcagctggacgccgttttgtctgcagcgaccgaaacctattccggtctgaccccggagcagaaagcgtacgttccggctatgttcaccgcagcactcaatatccaaaccagcgtcaataccgttgttcgtgattttgaaaattacgtgaagcagacgtgcaactcctcggcggtggtggataacaaactgaagatccaaaacgtgattatcgacgaatgttacggcgctccgggttctccgaccaacttggagtttatcaacactggcagcagcaaaggcaactgcgctattaaggcgctgatgcagctgactacaaaggcgaccacgcagatcgccccacgtcaggtggccggt

SEQ ID NO: 13 - DNA, 279 bp, synthetic construct
  source 1..279: mol_type = other DNA
atgtcaactacacaatatgatcacaaagaaagttgcaacggcttatattatcagggttcttgttatatcctgcacagcgactacaagtcttttgaggatgcgaaagctaactgcgcggcagaaagcagcaccctgccgaataagtccgacgtgttgaccacgtggctgatcgattacgtggaagatacctggggttccgacggcaacccgattaccaaaactacgagcgactaccaggatagcgacgtttcgcaagaggttcgtaaatacttctgcacc